European Patent Application EP 4 400 596 A1, published July 17, 2024. Title: NOVEL COMPOUND, USE OF SAID COMPOUND, PRODUCING METHOD THEREOF, COMPOSITION CONTAINING SAID COMPOUND, METHOD FOR PRODUCING OF 4-TREHALOSAMINE, AND MICROORGANISM. Applicant: 公益財団法人微生物化学研究会. Application JP. The sequence listing filed with the application follows.

SEQUENCE LISTING (3 sequences)

SEQ ID NO: 1 - DNA, 1446 bp, Streptomyces sp.
  source 1..1446: mol_type = genomic DNA
ggtgaacgctggcggcgtgcttaacacatgcaagtcgaacgatgaagcccttcggggtggattagtggcgaacgggtgagtaacacgtgggcaatctgcccttcactctgggacaagccctggaaacggggtctaataccggataatactcctgcctgcatgggtgggggttgaaagctccggcggtgaaggatgagcccgcggcctatcagcttgttggtggggtaatggcccaccaaggcgacgacgggtagccggcctgagagggcgaccggccacactgggactgagacacggcccagactcctacgggaggcagcagtggggaatattgcacaatgggcgaaagcctgatgcagcgacgccgcgtgagggatgacggccttcgggttgtaaacctctttcagcagggaagaagcgaaagtgacggtacctgcagaagaagcgccggctaactacgtgccagcagccgcggtaatacgtagggcgcaagcgttgtccggaattattgggcgtaaagagctcgtaggcggcttgtcacgtcggatgtgaaagcccgaggcttaacctcgggtctgcattcgatacgggctagctagagtgtggtaggggagatcggaattcctggtgtagcggtgaaatgcgcagatatcaggaggaacaccggtggcgaaggcggatctctgggccattactgacgctgaggagcgaaagcgtggggagcgaacaggattagataccctggtagtccacgccgtaaacgttgggaactaggtgttggcgacattccacgtcgtcggtgccgcagctaacgcattaagttccccgcctggggagtacggccgcaaggctaaaactcaaaggaattgacgggggcccgcacaagcagcggagcatgtggcttaattcgacgcaacgcgaagaaccttaccaaggcttgacatataccggaaagcattagagatagtgccccccttgtggtcggtatacaggtggtgcatggctgtcgtcagctcgtgtcgtgagatgttgggttaagtcccgcaacgagcgcaacccttgtcctgtgttgccagcatgcccttcggggtgatggggactcacaggagaccgccggggtcaactcggaggaaggtggggacgacgtcaagtcatcatgccccttatgtcttgggctgcacacgtgctacaatggccggtacaatgagctgcgataccgtgaggtggagcgaatctcaaaaagccggtctcagttcggattggggtctgcaactcgaccccatgaagttggagttgctagtaatcgcagatcagcattgctgcggtgaatacgttcccgggccttgtacacaccgcccgtcacgtcacgaaagtcggtaacacccgaagccggtggcccaacccgtaagggagggagctgtcgaaggtgggactggcgattgggac

SEQ ID NO: 2 - DNA, 31 bp, synthetic construct
  misc_feature 1..31: note = Primer of TREH1F
  source 1..31: mol_type = other DNA
ttagcggccgcgccaccatgccagggaggac

SEQ ID NO: 3 - DNA, 28 bp, synthetic construct
  misc_feature 1..28: note = Primer of TREH1R
  source 1..28: mol_type = other DNA
gggaattctcaccatggcaggaggctga